European Patent Specification EP 3 650 461 B1, published January 14, 2026. Title: NOVEL PEPTIDE EXHIBITING EFFECT OF RELEASING HEMATOPOIETIC STEM CELLS INTO BLOOD AND OSTEOPOROSIS THERAPEUTIC EFFECT AND USE THEREOF. Applicant: KYUNGPOOK NATIONAL UNIVERSITY INDUSTRY-ACADEMIC COOPERATION FOUNDATION. The sequence listing filed with the application follows.

SEQUENCE LISTING (16 sequences)

SEQ ID NO: 1 - protein, 8 aa, Artificial Sequence
  neuropeptide Y fragment(21-28)
YSALRHYI

SEQ ID NO: 2 - protein, 8 aa, Artificial Sequence
  neuropeptide Y fragment(24-31)
LRHYINLI

SEQ ID NO: 3 - protein, 8 aa, Artificial Sequence
  neuropeptide Y fragment(29-36)
NLITRQRY

SEQ ID NO: 4 - protein, 8 aa, Artificial Sequence
  neuropeptide Y fragment(21-28)
  MISC_FEATURE (5): Xaa is equal to D-amino acid of Arg
YSALXHYI

SEQ ID NO: 5 - protein, 8 aa, Artificial Sequence
  neuropeptide Y fragment(21-28)
  MISC_FEATURE (6): Xaa is equal to D-amino acid of His
YSALRXYI

SEQ ID NO: 6 - protein, 8 aa, Artificial Sequence
  neuropeptide Y fragment(21-28)
  MISC_FEATURE (5): Xaa is equal to D-amino acid of Arg
  MISC_FEATURE (6): Xaa is equal to D-amino acid of His
YSALXXYI

SEQ ID NO: 7 - protein, 16 aa, Artificial Sequence
  neuropeptide Y fragment(21-36)(Osteopep2)
YSALRHYINLITRQRY

SEQ ID NO: 8 - protein, 36 aa, Artificial Sequence
  neuropeptide Y(NPY)
YPSKPDNPGEDAPAEDMARYYSALRHYINLITRQRY

SEQ ID NO: 9 - DNA, 21 bp, Artificial Sequence
  SDF-1 alpha forward
ttcctatcagagcccatagag

SEQ ID NO: 10 - DNA, 20 bp, Artificial Sequence
  SDF-1 alpha reverse
ccagaccatcctggataatg

SEQ ID NO: 11 - DNA, 23 bp, Artificial Sequence
  Kit ligand(stem cell factor; SCF) forward
ccaaaagcaaagccaattacaag

SEQ ID NO: 12 - DNA, 20 bp, Artificial Sequence
  Kit ligand(stem cell factor; SCF) reverse
agactcgggcctacaatgga

SEQ ID NO: 13 - DNA, 18 bp, Artificial Sequence
  Angiopoietin-1 (Angpt1) forward
acgggggtcaattctaag

SEQ ID NO: 14 - DNA, 18 bp, Artificial Sequence
  Angiopoietin-1 (Angpt1) reverse
gccattcctgactccaca

SEQ ID NO: 15 - DNA, 21 bp, Artificial Sequence
  GAPDH forward
ttgctgttgaagtcgcaggag

SEQ ID NO: 16 - DNA, 20 bp, Artificial Sequence
  GAPDH reverse
tgtgtccgtcgtggatctga